European Patent Application EP 4 755 900 A1, published June 10, 2026. Title: An immunoanalytical method using Treponema pallidum antigen 17kDa (TpN17) as an antigen. Applicant: Denka Co. Ltd. The sequence listing filed with the application follows.

SEQUENCE LISTING (3 sequences)

SEQ ID NO: 1 - protein, 134 aa, Treponema pallidum
VSCTTVCPHAGKAKAEKVECALKGGIFRGTLPAADCPGIDTTVTFNADGTAQKVELALEKKSAPSPLTYRGTWMVREDGIVELSLVSSEQSKAPHEKELYELIDSNSVRYMGAPGAGKPSKEMAPFYVLKKTKK

SEQ ID NO: 2 - protein, 156 aa, Treponema pallidum
MKGSVRALCAFLGVGALGSALCVSCTTVCPHAGKAKAEKVECALKGGIFRGTLPAADCPGIDTTVTFNADGTAQKVELALEKKSAPSPLTYRGTWMVREDGIVELSLVSSEQSKAPHEKELYELIDSNSVRYMGAPGAGKPSKEMAPFYVLKKTKK

SEQ ID NO: 3 - protein, 123 aa, synthetic construct
  REGION 1..123: note = Synthetic
KAKAEKVECALKGGIFRGTLPAADCPGIDTTVTFNADGTAQKVELALEKKSAPSPLTYRGTWMVREDGIVELSLVSSEQSKAPHEKELYELIDSNSVRYMGAPGAGKPSKEMAPFYVLKKTKK